European Patent Application EP 4 667 057 A2, published December 24, 2025. Title: TRAILshort ANTIBODY AND METHODS OF USE. Applicant: Mayo Foundation for Medical Education and Research. Application EP, filed February 8, 2018. The sequence listing filed with the application follows.

SEQUENCE LISTING (32 sequences)

SEQ ID NO: 1 - protein, 10 aa, synthetic construct
  REGION 1..10: note = TRAILshort antibody VH CDR1 domain
GYIFTNNDMN

SEQ ID NO: 2 - protein, 17 aa, synthetic construct
  REGION 1..17: note = TRAILshort antibody VH CDR2 domain
GIDPGDGRTKYNEKFKG

SEQ ID NO: 3 - protein, 11 aa, synthetic construct
  REGION 1..11: note = TRAILshort antibody VH CDR3 domain
GRGGYEFGIDY

SEQ ID NO: 4 - protein, 118 aa, synthetic construct
  REGION 1..118: note = TRAILshort antibody VH domain
QVQLQQSGPELVKPGASVKISCKASGYIFTNNDMNWVKQRPGQGLEWIGGIDPGDGRTKYNEKFKGKATLTADKFSNTVYMQLSSLTSENSAVYFCGRGGYEFGIDYWGQGTSVTVSS

SEQ ID NO: 5 - protein, 118 aa, synthetic construct
  REGION 1..118: note = TRAILshort antibody VH domain
QVQLVQSGAEVKKPGATVKISCKVSGYIFTNNDMNWVQQAPGKGLEWMGGIDPGDGRTKYNEKFKGRVTITADESTSTAYMELSSLRSEDTAVYYCGRGGYEFGIDYWGQGTLVTVSS

SEQ ID NO: 6 - protein, 118 aa, synthetic construct
  REGION 1..118: note = TRAILshort antibody VH domain
QVQLVQSGAEVKKPGASVKVSCKASGYIFTNNDMNWVRQAPGQGLEWMGGIDPGDGRTKYNEKFKGRVTMTRDTSTNTVYMELSSLTSEDTAVYFCGRGGYEFGIDYWGQGTTVTVSS

SEQ ID NO: 7 - protein, 118 aa, synthetic construct
  REGION 1..118: note = TRAILshort antibody VH domain
QVQLVQSGAEVKKPGSSVKVSCKSSGYIFTNNDMNWVRQAPGQGLDWMGGIDPGDGRTKYNEKFKGRVTISADIFSNTAYMELNSLTSEDTAVYFCGRGGYEFGIDYWGQGTTVTVSS

SEQ ID NO: 8 - protein, 118 aa, synthetic construct
  REGION 1..118: note = TRAILshort antibody VH domain
QVQLVESGAEVKKPGASVKVSCKVSGYIFTNNDMNWVRQAPGEGLEWMGGIDPGDGRTKYNEKFKGRVTMTEDTSTDTAYMELSSLRSEDTAVYYCGRGGYEFGIDYWGQGTTVTVSS

SEQ ID NO: 9 - protein, 467 aa, synthetic construct
  REGION 1..467: note = TRAILshort antibody heavy chain
MGWTLVFLFLLSVTAGVHSQVQLQQSGPELVKPGASVKISCKASGYIFTNNDMNWVKQRPGQGLEWIGGIDPGDGRTKYNEKFKGKATLTADKFSNTVYMQLSSLTSENSAVYFCGRGGYEFGIDYWGQGTSVTVSSASTKGPSVFPLAPSSKSTSGGTAALGCLVKDYFPEPVTVSWNSGALTSGVHTFPAVLQSSGLYSLSSVVTVPSSSLGTQTYICNVNHKPSNTKVDKKVEPKSCDKTHTCPPCPAPELLGGPSVFLFPPKPKDTLMISRTPEVTCVVVDVSHEDPEVKFNWYVDGVEVHNAKTKPREEQYNSTYRVVSVLTVLHQDWLNGKEYKCKVSNKALPAPIEKTISKAKGQPREPQVYTLPPSRDELTKNQVSLTCLVKGFYPSDIAVEWESNGQPENNYKTTPPVLDSDGSFFLYSKLTVDKSRWQQGNVFSCSVMHEALHNHYTQKSLSLSPGK

SEQ ID NO: 10 - protein, 467 aa, synthetic construct
  REGION 1..467: note = TRAILshort antibody heavy chain
MGWTLVFLFLLSVTAGVHSQVQLVQSGAEVKKPGATVKISCKVSGYIFTNNDMNWVQQAPGKGLEWMGGIDPGDGRTKYNEKFKGRVTITADESTSTAYMELSSLRSEDTAVYYCGRGGYEFGIDYWGQGTLVTVSSASTKGPSVFPLAPSSKSTSGGTAALGCLVKDYFPEPVTVSWNSGALTSGVHTFPAVLQSSGLYSLSSVVTVPSSSLGTQTYICNVNHKPSNTKVDKKVEPKSCDKTHTCPPCPAPELLGGPSVFLFPPKPKDTLMISRTPEVTCVVVDVSHEDPEVKFNWYVDGVEVHNAKTKPREEQYNSTYRVVSVLTVLHQDWLNGKEYKCKVSNKALPAPIEKTISKAKGQPREPQVYTLPPSRDELTKNQVSLTCLVKGFYPSDIAVEWESNGQPENNYKTTPPVLDSDGSFFLYSKLTVDKSRWQQGNVFSCSVMHEALHNHYTQKSLSLSPGK

SEQ ID NO: 11 - protein, 467 aa, synthetic construct
  REGION 1..467: note = TRAILshort antibody heavy chain
MGWTLVFLFLLSVTAGVHSQVQLVQSGAEVKKPGASVKVSCKASGYIFTNNDMNWVRQAPGQGLEWMGGIDPGDGRTKYNEKFKGRVTMTRDTSTNTVYMELSSLTSEDTAVYFCGRGGYEFGIDYWGQGTTVTVSSASTKGPSVFPLAPSSKSTSGGTAALGCLVKDYFPEPVTVSWNSGALTSGVHTFPAVLQSSGLYSLSSVVTVPSSSLGTQTYICNVNHKPSNTKVDKKVEPKSCDKTHTCPPCPAPELLGGPSVFLFPPKPKDTLMISRTPEVTCVVVDVSHEDPEVKFNWYVDGVEVHNAKTKPREEQYNSTYRVVSVLTVLHQDWLNGKEYKCKVSNKALPAPIEKTISKAKGQPREPQVYTLPPSRDELTKNQVSLTCLVKGFYPSDIAVEWESNGQPENNYKTTPPVLDSDGSFFLYSKLTVDKSRWQQGNVFSCSVMHEALHNHYTQKSLSLSPGK

SEQ ID NO: 12 - protein, 467 aa, synthetic construct
  REGION 1..467: note = TRAILshort antibody heavy chain
MGWTLVFLFLLSVTAGVHSQVQLVQSGAEVKKPGSSVKVSCKSSGYIFTNNDMNWVRQAPGQGLDWMGGIDPGDGRTKYNEKFKGRVTISADIFSNTAYMELNSLTSEDTAVYFCGRGGYEFGIDYWGQGTTVTVSSASTKGPSVFPLAPSSKSTSGGTAALGCLVKDYFPEPVTVSWNSGALTSGVHTFPAVLQSSGLYSLSSVVTVPSSSLGTQTYICNVNHKPSNTKVDKKVEPKSCDKTHTCPPCPAPELLGGPSVFLFPPKPKDTLMISRTPEVTCVVVDVSHEDPEVKFNWYVDGVEVHNAKTKPREEQYNSTYRVVSVLTVLHQDWLNGKEYKCKVSNKALPAPIEKTISKAKGQPREPQVYTLPPSRDELTKNQVSLTCLVKGFYPSDIAVEWESNGQPENNYKTTPPVLDSDGSFFLYSKLTVDKSRWQQGNVFSCSVMHEALHNHYTQKSLSLSPGK

SEQ ID NO: 13 - protein, 467 aa, synthetic construct
  REGION 1..467: note = TRAILshort antibody heavy chain
MGWTLVFLFLLSVTAGVHSQVQLVESGAEVKKPGASVKVSCKVSGYIFTNNDMNWVRQAPGEGLEWMGGIDPGDGRTKYNEKFKGRVTMTEDTSTDTAYMELSSLRSEDTAVYYCGRGGYEFGIDYWGQGTTVTVSSASTKGPSVFPLAPSSKSTSGGTAALGCLVKDYFPEPVTVSWNSGALTSGVHTFPAVLQSSGLYSLSSVVTVPSSSLGTQTYICNVNHKPSNTKVDKKVEPKSCDKTHTCPPCPAPELLGGPSVFLFPPKPKDTLMISRTPEVTCVVVDVSHEDPEVKFNWYVDGVEVHNAKTKPREEQYNSTYRVVSVLTVLHQDWLNGKEYKCKVSNKALPAPIEKTISKAKGQPREPQVYTLPPSRDELTKNQVSLTCLVKGFYPSDIAVEWESNGQPENNYKTTPPVLDSDGSFFLYSKLTVDKSRWQQGNVFSCSVMHEALHNHYTQKSLSLSPGK

SEQ ID NO: 14 - protein, 17 aa, synthetic construct
  REGION 1..17: note = TRAILshort antibody VL CDR1 domain
KSSQSLLNSGNQKNSLA

SEQ ID NO: 15 - protein, 7 aa, synthetic construct
  REGION 1..7: note = TRAILshort antibody VL CDR2 domain
GASTRES

SEQ ID NO: 16 - protein, 9 aa, synthetic construct
  REGION 1..9: note = TRAILshort antibody VL CDR3 domain
QNDHSFPLT

SEQ ID NO: 17 - protein, 113 aa, synthetic construct
  REGION 1..113: note = TRAILshort antibody VL domain
DIVMTQSPSSLSVSAGEKVTMSCKSSQSLLNSGNQKNSLAWYQQKPGRPPTLLISGASTRESGVPDRFTGSGSGTDFTLTISSVQAEDLAVYYCQNDHSFPLTFGAGTKLELK

SEQ ID NO: 18 - protein, 113 aa, synthetic construct
  REGION 1..113: note = TRAILshort antibody VL domain
DVVMTQSPDSLAVSLGERATINCKSSQSLLNSGNQKNSLAWYQQKPGQPPKLLIYGASTRESGVPDRFSGSGSGTDFTLTISSLQAEDVAVYYCQNDHSFPLTFGQGTKLEIK

SEQ ID NO: 19 - protein, 113 aa, synthetic construct
  REGION 1..113: note = TRAILshort antibody VL domain
DIVMTQSPDSLAVSLGERATINCKSSQSLLNSGNQKNSLAWYQQKPGQPPKLLIYGASTRESGVPDRFSGSGSGTDFTLTISSLQAEDVAVYYCQNDHSFPLTFGGGTKLEIK

SEQ ID NO: 20 - protein, 113 aa, synthetic construct
  REGION 1..113: note = TRAILshort antibody VL domain
DIVMTQSPDSLAVSLGERATINCKSSQSLLNSGNQKNSLAWYQQRPGHPPKLLLYGASTRESGVPDRFSGSGSGTDFTLTISSLQAEDVAVYYCQNDHSFPLTFGGGTKVEIK

SEQ ID NO: 21 - protein, 113 aa, synthetic construct
  REGION 1..113: note = TRAILshort antibody VL domain
EIVLTQSPDSLAVSLGERATINCKSSQSLLNSGNQKNSLAWYQHKPGRPPKLLIYGASTRESGVPDRFSGSGSGEDFTLTISSLQAEDVAVYYCQNDHSFPLTFGPGTKVDLK

SEQ ID NO: 22 - protein, 240 aa, synthetic construct
  REGION 1..240: note = TRAILshort antibody light chain
MVSSAQFLGLLLLCFQGTRCDIVMTQSPSSLSVSAGEKVTMSCKSSQSLLNSGNQKNSLAWYQQKPGRPPTLLISGASTRESGVPDRFTGSGSGTDFTLTISSVQAEDLAVYYCQNDHSFPLTFGAGTKLELKRTVAAPSVFIFPPSDEQLKSGTASVVCLLNNFYPREAKVQWKVDNALQSGNSQESVTEQDSKDSTYSLSSTLTLSKADYEKHKVYACEVTHQGLSSPVTKSFNRGEC

SEQ ID NO: 23 - protein, 240 aa, synthetic construct
  REGION 1..240: note = TRAILshort antibody light chain
MVSSAQFLGLLLLCFQGTRCDVVMTQSPDSLAVSLGERATINCKSSQSLLNSGNQKNSLAWYQQKPGQPPKLLIYGASTRESGVPDRFSGSGSGTDFTLTISSLQAEDVAVYYCQNDHSFPLTFGQGTKLEIKRTVAAPSVFIFPPSDEQLKSGTASVVCLLNNFYPREAKVQWKVDNALQSGNSQESVTEQDSKDSTYSLSSTLTLSKADYEKHKVYACEVTHQGLSSPVTKSFNRGEC

SEQ ID NO: 24 - protein, 240 aa, synthetic construct
  REGION 1..240: note = TRAILshort antibody light chain
MVSSAQFLGLLLLCFQGTRCDIVMTQSPDSLAVSLGERATINCKSSQSLLNSGNQKNSLAWYQQKPGQPPKLLIYGASTRESGVPDRFSGSGSGTDFTLTISSLQAEDVAVYYCQNDHSFPLTFGGGTKLEIKRTVAAPSVFIFPPSDEQLKSGTASVVCLLNNFYPREAKVQWKVDNALQSGNSQESVTEQDSKDSTYSLSSTLTLSKADYEKHKVYACEVTHQGLSSPVTKSFNRGEC

SEQ ID NO: 25 - protein, 240 aa, synthetic construct
  REGION 1..240: note = TRAILshort antibody light chain
MVSSAQFLGLLLLCFQGTRCDIVMTQSPDSLAVSLGERATINCKSSQSLLNSGNQKNSLAWYQQRPGHPPKLLLYGASTRESGVPDRFSGSGSGTDFTLTISSLQAEDVAVYYCQNDHSFPLTFGGGTKVEIKRTVAAPSVFIFPPSDEQLKSGTASVVCLLNNFYPREAKVQWKVDNALQSGNSQESVTEQDSKDSTYSLSSTLTLSKADYEKHKVYACEVTHQGLSSPVTKSFNRGEC

SEQ ID NO: 26 - protein, 240 aa, synthetic construct
  REGION 1..240: note = TRAILshort antibody light chain
MVSSAQFLGLLLLCFQGTRCEIVLTQSPDSLAVSLGERATINCKSSQSLLNSGNQKNSLAWYQHKPGRPPKLLIYGASTRESGVPDRFSGSGSGEDFTLTISSLQAEDVAVYYCQNDHSFPLTFGPGTKVDLKRTVAAPSVFIFPPSDEQLKSGTASVVCLLNNFYPREAKVQWKVDNALQSGNSQESVTEQDSKDSTYSLSSTLTLSKADYEKHKVYACEVTHQGLSSPVTKSFNRGEC

SEQ ID NO: 27 - protein, 149 aa, Murine
MGWSWIILFLLSGTAGVHCQVQLQQSGPELVKPGASVKISCKASGYIFTNNDMNWVKQRPGQGLEWIGGIDPGDGRTKYNEKFKGKATLTADKFSNTVYMQLSSLTSENSAVYFCGRGGYEFGIDYWGQGTSVTVSSATTTAPSVYPLA

SEQ ID NO: 28 - protein, 163 aa, Murine
MVLMSLLFWVSGTCGDIVMTQSPSSLSVSAGEKVTMSCKSSQSLLNSGNQKNSLAWYQQKPGRPPTLLISGASTRESGVPDRFTGSGSGTDFTLTISSVQAEDLAVYYCQNDHSFPLTFGAGTKLELKRADAAPTVSIFPPSSEQLTSGGASVVCFLNNFYPK

SEQ ID NO: 29 - protein, 330 aa, Homo sapiens [sequence omitted]

SEQ ID NO: 30 - protein, 106 aa, Homo sapiens
TVAAPSVFIFPPSDEQLKSGTASVVCLLNNFYPREAKVQWKVDNALQSGNSQESVTEQDSKDSTYSLSSTLTLSKADYEKHKVYACEVTHQGLSSPVTKSFNRGEC

SEQ ID NO: 31 - DNA, 41 bp, synthetic construct
  misc_feature 1..41: note = oligonucleotide probe
  source 1..41: mol_type = other DNA
tcgttagaaagactccaagaatgaaaaggctctgggccgca

SEQ ID NO: 32 - protein, 101 aa, Homo sapiens
MAMMEVQGGPSLGQTCVLIVIFTVLLQSLCVAVTYVYFTNELKQMQDKYSKSGIACFLKEDDSYWDPNDEESMNSPCWQVKWQLRQLVRKTPRMKRLWAAK